European Patent Application EP 4 506 364 A1, published February 12, 2025. Title: ANTIGEN BINDING PROTEIN TARGETING CD40, AND PREPARATION THEREFOR AND USE THEREOF. Applicant: HARBOUR BIOMED (SHANGHAI) CO., LTD. Application EP. The sequence listing filed with the application follows.

SEQUENCE LISTING (143 sequences)

SEQ ID NO: 1 - protein, 25 aa, synthetic construct [sequence omitted]

SEQ ID NO: 2 - protein, 25 aa, synthetic construct
QVQLVESGGGVVQPGRSLRLSCAAS

SEQ ID NO: 3 - protein, 25 aa, synthetic construct
QVQLVESGGGVVQPGKSLRLSCAAS

SEQ ID NO: 4 - protein, 7 aa, synthetic construct
GYTFTGY

SEQ ID NO: 5 - protein, 7 aa, synthetic construct
GFSFSST

SEQ ID NO: 6 - protein, 7 aa, synthetic construct
GFTFSSN

SEQ ID NO: 7 - protein, 7 aa, synthetic construct
GYTFAGY

SEQ ID NO: 8 - protein, 19 aa, synthetic construct
YMHWVRQAPGQGLEWMGWI

SEQ ID NO: 9 - protein, 19 aa, synthetic construct
YVCWVRQAPGKGLEWIACI

SEQ ID NO: 10 - protein, 19 aa, synthetic construct
GIHWVRQAPGKGLEWVAVI

SEQ ID NO: 11 - protein, 19 aa, synthetic construct
YMYWVRQAPGQGLEWMGWI

SEQ ID NO: 12 - protein, 6 aa, synthetic construct
NPDSGG

SEQ ID NO: 13 - protein, 6 aa, synthetic construct
YTGDGT

SEQ ID NO: 14 - protein, 6 aa, synthetic construct
WSDGSN

SEQ ID NO: 15 - protein, 6 aa, synthetic construct
NPDSGA

SEQ ID NO: 16 - protein, 41 aa, synthetic construct
TNYAQKFQGRVTMTRDTSISTAYMELNRLRSDDTAVYYCAR

SEQ ID NO: 17 - protein, 41 aa, synthetic construct
NYSASWAKGRFTISKDSSKNTVYLQMNSLRAEDTAVYFCAR

SEQ ID NO: 18 - protein, 41 aa, synthetic construct
KFYADSVKGRFTISRDNSKNTLYLQMNSLRAEDTAVYYCAR

SEQ ID NO: 19 - protein, 41 aa, synthetic construct
PTYAQKFQGRVTMTRDTSISTAYMELSRLRSDDTAVYYCAR

SEQ ID NO: 20 - protein, 17 aa, synthetic construct
DQPLGYCTNGVCSYFDY

SEQ ID NO: 21 - protein, 11 aa, synthetic construct
PDITYGFAINF

SEQ ID NO: 22 - protein, 13 aa, synthetic construct
ASGSGSYYNFFDY

SEQ ID NO: 23 - protein, 16 aa, synthetic construct
EKIYYGSGNYYPSFDY

SEQ ID NO: 24 - protein, 11 aa, synthetic construct
WGQGTLVTVSS

SEQ ID NO: 25 - protein, 11 aa, synthetic construct
WGPGTLVTVSS

SEQ ID NO: 26 - protein, 23 aa, synthetic construct
DIQMTQSPSSVSASVGDRVTITC

SEQ ID NO: 27 - protein, 23 aa, synthetic construct
DIQMTQSPSSLSASVGDRVTIKC

SEQ ID NO: 28 - protein, 23 aa, synthetic construct
EIVMTQSPATLSVSPGERATLSC

SEQ ID NO: 29 - protein, 23 aa, synthetic construct
DIQLTQSPSFLSASVGDRVTITC

SEQ ID NO: 30 - protein, 11 aa, synthetic construct
RASQGIYSWLA

SEQ ID NO: 31 - protein, 11 aa, synthetic construct
QASQSISSRLA

SEQ ID NO: 32 - protein, 11 aa, synthetic construct
RASQSVRSNLA

SEQ ID NO: 33 - protein, 11 aa, synthetic construct
RASQGISSYLA

SEQ ID NO: 34 - protein, 15 aa, synthetic construct
WYQQKPGKAPNLLIY

SEQ ID NO: 35 - protein, 15 aa, synthetic construct
WYQQKPGKPPKLLIY

SEQ ID NO: 36 - protein, 15 aa, synthetic construct
WYQQKPGQAPRLLIY

SEQ ID NO: 37 - protein, 15 aa, synthetic construct
WYQQKPGKAPKLLIY

SEQ ID NO: 38 - protein, 7 aa, synthetic construct
TASTLQS

SEQ ID NO: 39 - protein, 7 aa, synthetic construct
RASTLAS

SEQ ID NO: 40 - protein, 7 aa, synthetic construct
GASTRAT

SEQ ID NO: 41 - protein, 7 aa, synthetic construct
AASTLQS

SEQ ID NO: 42 - protein, 32 aa, synthetic construct
GVPSRFSGSGSGTDFTLTISSLQPEDFATYYC

SEQ ID NO: 43 - protein, 32 aa, synthetic construct
GVPSRFSGSGSGTDFTLTISSLQPEDVATYYC

SEQ ID NO: 44 - protein, 32 aa, synthetic construct
GIPARFSGSGSGTEFTLTINSLQSEDFAVYYC

SEQ ID NO: 45 - protein, 32 aa, synthetic construct
GVPSRFSGSGSGTEFTLTISSLQPEDFATYYC

SEQ ID NO: 46 - protein, 9 aa, synthetic construct
QQANIFPLT

SEQ ID NO: 47 - protein, 10 aa, synthetic construct
QCTGYGISWP

SEQ ID NO: 48 - protein, 8 aa, synthetic construct
QQHNKWIT

SEQ ID NO: 49 - protein, 9 aa, synthetic construct
QQLNSYPWT

SEQ ID NO: 50 - protein, 9 aa, synthetic construct
QQLESYPWT

SEQ ID NO: 51 - protein, 9 aa, synthetic construct
QQLLSYPWT

SEQ ID NO: 52 - protein, 9 aa, synthetic construct
QQLTSYPWT

SEQ ID NO: 53 - protein, 9 aa, synthetic construct
QQLASYPWT

SEQ ID NO: 54 - protein, 9 aa, synthetic construct
QQLFSYPWT

SEQ ID NO: 55 - protein, 9 aa, synthetic construct
QQLYSYPWT

SEQ ID NO: 56 - protein, 9 aa, synthetic construct
QQLISYPWT

SEQ ID NO: 57 - protein, 9 aa, synthetic construct
QQLWSYPWT

SEQ ID NO: 58 - protein, 9 aa, synthetic construct
QQLMSYPWT

SEQ ID NO: 59 - protein, 9 aa, synthetic construct
QQLQSYPWT

SEQ ID NO: 60 - protein, 9 aa, synthetic construct
QQLDSYPWT

SEQ ID NO: 61 - protein, 9 aa, synthetic construct
QQLGSYPWT

SEQ ID NO: 62 - protein, 9 aa, synthetic construct
QQLVSYPWT

SEQ ID NO: 63 - protein, 9 aa, synthetic construct
QQLNIYPWT

SEQ ID NO: 64 - protein, 9 aa, synthetic construct
QQLNFYPWT

SEQ ID NO: 65 - protein, 9 aa, synthetic construct
QQLNEYPWT

SEQ ID NO: 66 - protein, 9 aa, synthetic construct
QQLNLYPWT

SEQ ID NO: 67 - protein, 9 aa, synthetic construct
QQLNRYPWT

SEQ ID NO: 68 - protein, 9 aa, synthetic construct
QQLNNYPWT

SEQ ID NO: 69 - protein, 9 aa, synthetic construct
QQLNTYPWT

SEQ ID NO: 70 - protein, 9 aa, synthetic construct
QQLNQYPWT

SEQ ID NO: 71 - protein, 9 aa, synthetic construct
QQLNVYPWT

SEQ ID NO: 72 - protein, 9 aa, synthetic construct
QQLNMYPWT

SEQ ID NO: 73 - protein, 9 aa, synthetic construct
QQLNHYPWT

SEQ ID NO: 74 - protein, 10 aa, synthetic construct
FGGGTKVEIK

SEQ ID NO: 75 - protein, 10 aa, synthetic construct
IGGGTKVEIK

SEQ ID NO: 76 - protein, 10 aa, synthetic construct
FGQGTRLEIK

SEQ ID NO: 77 - protein, 10 aa, synthetic construct
FGQGTKVEIK

SEQ ID NO: 78 - protein, 126 aa, synthetic construct
QVQLVQSGAEVKKPGASVKVSCKASGYTFTGYYMHWVRQAPGQGLEWMGWINPDSGGTNYAQKFQGRVTMTRDTSISTAYMELNRLRSDDTAVYYCARDQPLGYCTNGVCSYFDYWGQGTLVTVSS

SEQ ID NO: 79 - protein, 120 aa, synthetic construct
QVQLVESGGGVVQPGRSLRLSCAASGFSFSSTYVCWVRQAPGKGLEWIACIYTGDGTNYSASWAKGRFTISKDSSKNTVYLQMNSLRAEDTAVYFCARPDITYGFAINFWGPGTLVTVSS

SEQ ID NO: 80 - protein, 122 aa, synthetic construct
QVQLVESGGGVVQPGKSLRLSCAASGFTFSSNGIHWVRQAPGKGLEWVAVIWSDGSNKFYADSVKGRFTISRDNSKNTLYLQMNSLRAEDTAVYYCARASGSGSYYNFFDYWGQGTLVTVSS

SEQ ID NO: 81 - protein, 125 aa, synthetic construct
QVQLVQSGAEVKKPGASVKVSCKASGYTFAGYYMYWVRQAPGQGLEWMGWINPDSGAPTYAQKFQGRVTMTRDTSISTAYMELSRLRSDDTAVYYCAREKIYYGSGNYYPSFDYWGQGTLVTVSS

SEQ ID NO: 82 - protein, 107 aa, synthetic construct
DIQMTQSPSSVSASVGDRVTITCRASQGIYSWLAWYQQKPGKAPNLLIYTASTLQSGVPSRFSGSGSGTDFTLTISSLQPEDFATYYCQQANIFPLTFGGGTKVEIK

SEQ ID NO: 83 - protein, 108 aa, synthetic construct
DIQMTQSPSSLSASVGDRVTIKCQASQSISSRLAWYQQKPGKPPKLLIYRASTLASGVPSRFSGSGSGTDFTLTISSLQPEDVATYYCQCTGYGISWPIGGGTKVEIK

SEQ ID NO: 84 - protein, 106 aa, synthetic construct
EIVMTQSPATLSVSPGERATLSCRASQSVRSNLAWYQQKPGQAPRLLIYGASTRATGIPARFSGSGSGTEFTLTINSLQSEDFAVYYCQQHNKWITFGQGTRLEIK

SEQ ID NO: 85 - protein, 107 aa, synthetic construct
DIQLTQSPSFLSASVGDRVTITCRASQGISSYLAWYQQKPGKAPKLLIYAASTLQSGVPSRFSGSGSGTEFTLTISSLQPEDFATYYCQQLNSYPWTFGQGTKVEIK

SEQ ID NO: 86 - protein, 107 aa, synthetic construct
DIQLTQSPSFLSASVGDRVTITCRASQGISSYLAWYQQKPGKAPKLLIYAASTLQSGVPSRFSGSGSGTEFTLTISSLQPEDFATYYCQQLESYPWTFGQGTKVEIK

SEQ ID NO: 87 - protein, 107 aa, synthetic construct
DIQLTQSPSFLSASVGDRVTITCRASQGISSYLAWYQQKPGKAPKLLIYAASTLQSGVPSRFSGSGSGTEFTLTISSLQPEDFATYYCQQLLSYPWTFGQGTKVEIK

SEQ ID NO: 88 - protein, 107 aa, synthetic construct
DIQLTQSPSFLSASVGDRVTITCRASQGISSYLAWYQQKPGKAPKLLIYAASTLQSGVPSRFSGSGSGTEFTLTISSLQPEDFATYYCQQLTSYPWTFGQGTKVEIK

SEQ ID NO: 89 - protein, 107 aa, synthetic construct
DIQLTQSPSFLSASVGDRVTITCRASQGISSYLAWYQQKPGKAPKLLIYAASTLQSGVPSRFSGSGSGTEFTLTISSLQPEDFATYYCQQLASYPWTFGQGTKVEIK

SEQ ID NO: 90 - protein, 107 aa, synthetic construct
DIQLTQSPSFLSASVGDRVTITCRASQGISSYLAWYQQKPGKAPKLLIYAASTLQSGVPSRFSGSGSGTEFTLTISSLQPEDFATYYCQQLFSYPWTFGQGTKVEIK

SEQ ID NO: 91 - protein, 107 aa, synthetic construct
DIQLTQSPSFLSASVGDRVTITCRASQGISSYLAWYQQKPGKAPKLLIYAASTLQSGVPSRFSGSGSGTEFTLTISSLQPEDFATYYCQQLYSYPWTFGQGTKVEIK

SEQ ID NO: 92 - protein, 107 aa, synthetic construct
DIQLTQSPSFLSASVGDRVTITCRASQGISSYLAWYQQKPGKAPKLLIYAASTLQSGVPSRFSGSGSGTEFTLTISSLQPEDFATYYCQQLISYPWTFGQGTKVEIK

SEQ ID NO: 93 - protein, 107 aa, synthetic construct
DIQLTQSPSFLSASVGDRVTITCRASQGISSYLAWYQQKPGKAPKLLIYAASTLQSGVPSRFSGSGSGTEFTLTISSLQPEDFATYYCQQLWSYPWTFGQGTKVEIK

SEQ ID NO: 94 - protein, 107 aa, synthetic construct
DIQLTQSPSFLSASVGDRVTITCRASQGISSYLAWYQQKPGKAPKLLIYAASTLQSGVPSRFSGSGSGTEFTLTISSLQPEDFATYYCQQLMSYPWTFGQGTKVEIK

SEQ ID NO: 95 - protein, 107 aa, synthetic construct
DIQLTQSPSFLSASVGDRVTITCRASQGISSYLAWYQQKPGKAPKLLIYAASTLQSGVPSRFSGSGSGTEFTLTISSLQPEDFATYYCQQLQSYPWTFGQGTKVEIK

SEQ ID NO: 96 - protein, 107 aa, synthetic construct
DIQLTQSPSFLSASVGDRVTITCRASQGISSYLAWYQQKPGKAPKLLIYAASTLQSGVPSRFSGSGSGTEFTLTISSLQPEDFATYYCQQLDSYPWTFGQGTKVEIK

SEQ ID NO: 97 - protein, 107 aa, synthetic construct
DIQLTQSPSFLSASVGDRVTITCRASQGISSYLAWYQQKPGKAPKLLIYAASTLQSGVPSRFSGSGSGTEFTLTISSLQPEDFATYYCQQLGSYPWTFGQGTKVEIK

SEQ ID NO: 98 - protein, 107 aa, synthetic construct
DIQLTQSPSFLSASVGDRVTITCRASQGISSYLAWYQQKPGKAPKLLIYAASTLQSGVPSRFSGSGSGTEFTLTISSLQPEDFATYYCQQLVSYPWTFGQGTKVEIK

SEQ ID NO: 99 - protein, 107 aa, synthetic construct
DIQLTQSPSFLSASVGDRVTITCRASQGISSYLAWYQQKPGKAPKLLIYAASTLQSGVPSRFSGSGSGTEFTLTISSLQPEDFATYYCQQLNIYPWTFGQGTKVEIK

SEQ ID NO: 100 - protein, 107 aa, synthetic construct
DIQLTQSPSFLSASVGDRVTITCRASQGISSYLAWYQQKPGKAPKLLIYAASTLQSGVPSRFSGSGSGTEFTLTISSLQPEDFATYYCQQLNFYPWTFGQGTKVEIK

SEQ ID NO: 101 - protein, 107 aa, synthetic construct
DIQLTQSPSFLSASVGDRVTITCRASQGISSYLAWYQQKPGKAPKLLIYAASTLQSGVPSRFSGSGSGTEFTLTISSLQPEDFATYYCQQLNEYPWTFGQGTKVEIK

SEQ ID NO: 102 - protein, 107 aa, synthetic construct
DIQLTQSPSFLSASVGDRVTITCRASQGISSYLAWYQQKPGKAPKLLIYAASTLQSGVPSRFSGSGSGTEFTLTISSLQPEDFATYYCQQLNLYPWTFGQGTKVEIK

SEQ ID NO: 103 - protein, 107 aa, synthetic construct
DIQLTQSPSFLSASVGDRVTITCRASQGISSYLAWYQQKPGKAPKLLIYAASTLQSGVPSRFSGSGSGTEFTLTISSLQPEDFATYYCQQLNRYPWTFGQGTKVEIK

SEQ ID NO: 104 - protein, 107 aa, synthetic construct
DIQLTQSPSFLSASVGDRVTITCRASQGISSYLAWYQQKPGKAPKLLIYAASTLQSGVPSRFSGSGSGTEFTLTISSLQPEDFATYYCQQLNNYPWTFGQGTKVEIK

SEQ ID NO: 105 - protein, 107 aa, synthetic construct
DIQLTQSPSFLSASVGDRVTITCRASQGISSYLAWYQQKPGKAPKLLIYAASTLQSGVPSRFSGSGSGTEFTLTISSLQPEDFATYYCQQLNTYPWTFGQGTKVEIK

SEQ ID NO: 106 - protein, 107 aa, synthetic construct
DIQLTQSPSFLSASVGDRVTITCRASQGISSYLAWYQQKPGKAPKLLIYAASTLQSGVPSRFSGSGSGTEFTLTISSLQPEDFATYYCQQLNQYPWTFGQGTKVEIK

SEQ ID NO: 107 - protein, 107 aa, synthetic construct
DIQLTQSPSFLSASVGDRVTITCRASQGISSYLAWYQQKPGKAPKLLIYAASTLQSGVPSRFSGSGSGTEFTLTISSLQPEDFATYYCQQLNVYPWTFGQGTKVEIK

SEQ ID NO: 108 - protein, 107 aa, synthetic construct
DIQLTQSPSFLSASVGDRVTITCRASQGISSYLAWYQQKPGKAPKLLIYAASTLQSGVPSRFSGSGSGTEFTLTISSLQPEDFATYYCQQLNMYPWTFGQGTKVEIK

SEQ ID NO: 109 - protein, 107 aa, synthetic construct
DIQLTQSPSFLSASVGDRVTITCRASQGISSYLAWYQQKPGKAPKLLIYAASTLQSGVPSRFSGSGSGTEFTLTISSLQPEDFATYYCQQLNHYPWTFGQGTKVEIK

SEQ ID NO: 110 - protein, 452 aa, synthetic construct
QVQLVQSGAEVKKPGASVKVSCKASGYTFTGYYMHWVRQAPGQGLEWMGWINPDSGGTNYAQKFQGRVTMTRDTSISTAYMELNRLRSDDTAVYYCARDQPLGYCTNGVCSYFDYWGQGTLVTVSSASTKGPSVFPLAPCSRSTSESTAALGCLVKDYFPEPVTVSWNSGALTSGVHTFPAVLQSSGLYSLSSVVTVPSSNFGTQTYTCNVDHKPSNTKVDKTVERKCCVECPPCPAPPVAGPSVFLFPPKPKDTLMISRTPEVTCVVVDVSHEDPEVQFNWYVDGVEVHNAKTKPREEQFNSTFRVVSVLTVVHQDWLNGKEYKCKVSNKGLPAPIEKTISKTKGQPREPQVYTLPPSREEMTKNQVSLTCLVKGFYPSDIAVEWESNGQPENNYKTTPPMLDSDGSFFLYSKLTVDKSRWQQGNVFSCSVMHEALHNHYTQKSLSLSPGK

SEQ ID NO: 111 - protein, 450 aa, synthetic construct
QVQLVESGGGVVQPGRSLRLSCAASGFSFSSTYVCWVRQAPGKGLEWIACIYTGDGTNYSASWAKGRFTISKDSSKNTVYLQMNSLRAEDTAVYFCARPDITYGFAINFWGPGTLVTVSSASTKGPSVFPLAPSSKSTSGGTAALGCLVKDYFPEPVTVSWNSGALTSGVHTFPAVLQSSGLYSLSSVVTVPSSSLGTQTYICNVNHKPSNTKVDKKVEPKSCDKTHTCPPCPAPELLGGPSVFLFPPKPKDTLMISRTPEVTCVVVDVSHEDPEVKFNWYVDGVEVHNAKTKPREEQYNSTYRVVSVLTVLHQDWLNGKEYKCKVSNKALPAPIEKTISKAKGQPREPQVYTLPPSREEMTKNQVSLTCLVKGFYPSDIAVEWESNGQPENNYKTTPPVLDSDGSFFLYSKLTVDKSRWQQGNVFSCSVMHEALHNHYTQKSLSLSPGK

SEQ ID NO: 112 - protein, 450 aa, synthetic construct
QVQLVESGGGVVQPGRSLRLSCAASGFSFSSTYVCWVRQAPGKGLEWIACIYTGDGTNYSASWAKGRFTISKDSSKNTVYLQMNSLRAEDTAVYFCARPDITYGFAINFWGPGTLVTVSSASTKGPSVFPLAPSSKSTSGGTAALGCLVKDYFPEPVTVSWNSGALTSGVHTFPAVLQSSGLYSLSSVVTVPSSSLGTQTYICNVNHKPSNTKVDKKVEPKSCDKTHTCPPCPAPELLGGPSVFLFPPKPKDTLMISRTPEVTCVVVDVEHEDPEVKFNWYVDGVEVHNAKTKPREEQYNSTYRVVSVLTVLHQDWLNGKEYKCKVSNKALPAPIEKTISKAKGQPREPQVYTLPPSREEMTKNQVSLTCLVKGFYPSDIAVEWESNGQPENNYKTTPPVLDSDGSFFLYSKLTVDKSRWQQGNVFSCSVMHEALHNHYTQKSLSLSPGK

SEQ ID NO: 113 - protein, 448 aa, synthetic construct
QVQLVESGGGVVQPGKSLRLSCAASGFTFSSNGIHWVRQAPGKGLEWVAVIWSDGSNKFYADSVKGRFTISRDNSKNTLYLQMNSLRAEDTAVYYCARASGSGSYYNFFDYWGQGTLVTVSSASTKGPSVFPLAPCSRSTSESTAALGCLVKDYFPEPVTVSWNSGALTSGVHTFPAVLQSSGLYSLSSVVTVPSSNFGTQTYTCNVDHKPSNTKVDKTVERKCCVECPPCPAPPVAGPSVFLFPPKPKDTLMISRTPEVTCVVVDVSHEDPEVQFNWYVDGVEVHNAKTKPREEQFNSTFRVVSVLTVVHQDWLNGKEYKCKVSNKGLPAPIEKTISKTKGQPREPQVYTLPPSREEMTKNQVSLTCLVKGFYPSDIAVEWESNGQPENNYKTTPPMLDSDGSFFLYSKLTVDKSRWQQGNVFSCSVMHEALHNHYTQKSLSLSPGK

SEQ ID NO: 114 - protein, 451 aa, synthetic construct
QVQLVQSGAEVKKPGASVKVSCKASGYTFAGYYMYWVRQAPGQGLEWMGWINPDSGAPTYAQKFQGRVTMTRDTSISTAYMELSRLRSDDTAVYYCAREKIYYGSGNYYPSFDYWGQGTLVTVSSASTKGPSVFPLAPCSRSTSESTAALGCLVKDYFPEPVTVSWNSGALTSGVHTFPAVLQSSGLYSLSSVVTVPSSNFGTQTYTCNVDHKPSNTKVDKTVERKCCVECPPCPAPPVAGPSVFLFPPKPKDTLMISRTPEVTCVVVDVSHEDPEVQFNWYVDGVEVHNAKTKPREEQFNSTFRVVSVLTVVHQDWLNGKEYKCKVSNKGLPAPIEKTISKTKGQPREPQVYTLPPSREEMTKNQVSLTCLVKGFYPSDIAVEWESNGQPENNYKTTPPMLDSDGSFFLYSKLTVDKSRWQQGNVFSCSVMHEALHNHYTQKSLSLSPGK

SEQ ID NO: 115 - protein, 455 aa, synthetic construct
QVQLVQSGAEVKKPGASVKVSCKASGYTFAGYYMYWVRQAPGQGLEWMGWINPDSGAPTYAQKFQGRVTMTRDTSISTAYMELSRLRSDDTAVYYCAREKIYYGSGNYYPSFDYWGQGTLVTVSSASTKGPSVFPLAPSSKSTSGGTAALGCLVKDYFPEPVTVSWNSGALTSGVHTFPAVLQSSGLYSLSSVVTVPSSSLGTQTYICNVNHKPSNTKVDKKVEPKSCDKTHTCPPCPAPEAAGAPSVFLFPPKPKDTLMISRTPEVTCVVVDVSHEDPEVKFNWYVDGVEVHNAKTKPREEQYNSTYRVVSVLTVLHQDWLNGKEYKCKVSNKALPAPIEKTISKAKGQPREPQVYTLPPSREEMTKNQVSLTCLVKGFYPSDIAVEWESNGQPENNYKTTPPVLDSDGSFFLYSKLTVDKSRWQQGNVFSCSVMHEALHNHYTQKSLSLSPGK

SEQ ID NO: 116 - protein, 214 aa, synthetic construct
DIQMTQSPSSVSASVGDRVTITCRASQGIYSWLAWYQQKPGKAPNLLIYTASTLQSGVPSRFSGSGSGTDFTLTISSLQPEDFATYYCQQANIFPLTFGGGTKVEIKRTVAAPSVFIFPPSDEQLKSGTASVVCLLNNFYPREAKVQWKVDNALQSGNSQESVTEQDSKDSTYSLSSTLTLSKADYEKHKVYACEVTHQGLSSPVTKSFNRGEC

SEQ ID NO: 117 - protein, 215 aa, synthetic construct
DIQMTQSPSSLSASVGDRVTIKCQASQSISSRLAWYQQKPGKPPKLLIYRASTLASGVPSRFSGSGSGTDFTLTISSLQPEDVATYYCQCTGYGISWPIGGGTKVEIKRTVAAPSVFIFPPSDEQLKSGTASVVCLLNNFYPREAKVQWKVDNALQSGNSQESVTEQDSKDSTYSLSSTLTLSKADYEKHKVYACEVTHQGLSSPVTKSFNRGEC

SEQ ID NO: 118 - protein, 213 aa, synthetic construct
EIVMTQSPATLSVSPGERATLSCRASQSVRSNLAWYQQKPGQAPRLLIYGASTRATGIPARFSGSGSGTEFTLTINSLQSEDFAVYYCQQHNKWITFGQGTRLEIKRTVAAPSVFIFPPSDEQLKSGTASVVCLLNNFYPREAKVQWKVDNALQSGNSQESVTEQDSKDSTYSLSSTLTLSKADYEKHKVYACEVTHQGLSSPVTKSFNRGEC

SEQ ID NO: 119 - protein, 214 aa, synthetic construct
DIQLTQSPSFLSASVGDRVTITCRASQGISSYLAWYQQKPGKAPKLLIYAASTLQSGVPSRFSGSGSGTEFTLTISSLQPEDFATYYCQQLNSYPWTFGQGTKVEIKRTVAAPSVFIFPPSDEQLKSGTASVVCLLNNFYPREAKVQWKVDNALQSGNSQESVTEQDSKDSTYSLSSTLTLSKADYEKHKVYACEVTHQGLSSPVTKSFNRGEC

SEQ ID NO: 120 - protein, 214 aa, synthetic construct
DIQLTQSPSFLSASVGDRVTITCRASQGISSYLAWYQQKPGKAPKLLIYAASTLQSGVPSRFSGSGSGTEFTLTISSLQPEDFATYYCQQLESYPWTFGQGTKVEIKRTVAAPSVFIFPPSDEQLKSGTASVVCLLNNFYPREAKVQWKVDNALQSGNSQESVTEQDSKDSTYSLSSTLTLSKADYEKHKVYACEVTHQGLSSPVTKSFNRGEC

SEQ ID NO: 121 - protein, 214 aa, synthetic construct
DIQLTQSPSFLSASVGDRVTITCRASQGISSYLAWYQQKPGKAPKLLIYAASTLQSGVPSRFSGSGSGTEFTLTISSLQPEDFATYYCQQLLSYPWTFGQGTKVEIKRTVAAPSVFIFPPSDEQLKSGTASVVCLLNNFYPREAKVQWKVDNALQSGNSQESVTEQDSKDSTYSLSSTLTLSKADYEKHKVYACEVTHQGLSSPVTKSFNRGEC

SEQ ID NO: 122 - protein, 214 aa, synthetic construct
DIQLTQSPSFLSASVGDRVTITCRASQGISSYLAWYQQKPGKAPKLLIYAASTLQSGVPSRFSGSGSGTEFTLTISSLQPEDFATYYCQQLTSYPWTFGQGTKVEIKRTVAAPSVFIFPPSDEQLKSGTASVVCLLNNFYPREAKVQWKVDNALQSGNSQESVTEQDSKDSTYSLSSTLTLSKADYEKHKVYACEVTHQGLSSPVTKSFNRGEC

SEQ ID NO: 123 - protein, 214 aa, synthetic construct
DIQLTQSPSFLSASVGDRVTITCRASQGISSYLAWYQQKPGKAPKLLIYAASTLQSGVPSRFSGSGSGTEFTLTISSLQPEDFATYYCQQLASYPWTFGQGTKVEIKRTVAAPSVFIFPPSDEQLKSGTASVVCLLNNFYPREAKVQWKVDNALQSGNSQESVTEQDSKDSTYSLSSTLTLSKADYEKHKVYACEVTHQGLSSPVTKSFNRGEC

SEQ ID NO: 124 - protein, 214 aa, synthetic construct
DIQLTQSPSFLSASVGDRVTITCRASQGISSYLAWYQQKPGKAPKLLIYAASTLQSGVPSRFSGSGSGTEFTLTISSLQPEDFATYYCQQLFSYPWTFGQGTKVEIKRTVAAPSVFIFPPSDEQLKSGTASVVCLLNNFYPREAKVQWKVDNALQSGNSQESVTEQDSKDSTYSLSSTLTLSKADYEKHKVYACEVTHQGLSSPVTKSFNRGEC

SEQ ID NO: 125 - protein, 214 aa, synthetic construct
DIQLTQSPSFLSASVGDRVTITCRASQGISSYLAWYQQKPGKAPKLLIYAASTLQSGVPSRFSGSGSGTEFTLTISSLQPEDFATYYCQQLYSYPWTFGQGTKVEIKRTVAAPSVFIFPPSDEQLKSGTASVVCLLNNFYPREAKVQWKVDNALQSGNSQESVTEQDSKDSTYSLSSTLTLSKADYEKHKVYACEVTHQGLSSPVTKSFNRGEC

SEQ ID NO: 126 - protein, 214 aa, synthetic construct
DIQLTQSPSFLSASVGDRVTITCRASQGISSYLAWYQQKPGKAPKLLIYAASTLQSGVPSRFSGSGSGTEFTLTISSLQPEDFATYYCQQLISYPWTFGQGTKVEIKRTVAAPSVFIFPPSDEQLKSGTASVVCLLNNFYPREAKVQWKVDNALQSGNSQESVTEQDSKDSTYSLSSTLTLSKADYEKHKVYACEVTHQGLSSPVTKSFNRGEC

SEQ ID NO: 127 - protein, 214 aa, synthetic construct
DIQLTQSPSFLSASVGDRVTITCRASQGISSYLAWYQQKPGKAPKLLIYAASTLQSGVPSRFSGSGSGTEFTLTISSLQPEDFATYYCQQLWSYPWTFGQGTKVEIKRTVAAPSVFIFPPSDEQLKSGTASVVCLLNNFYPREAKVQWKVDNALQSGNSQESVTEQDSKDSTYSLSSTLTLSKADYEKHKVYACEVTHQGLSSPVTKSFNRGEC

SEQ ID NO: 128 - protein, 214 aa, synthetic construct
DIQLTQSPSFLSASVGDRVTITCRASQGISSYLAWYQQKPGKAPKLLIYAASTLQSGVPSRFSGSGSGTEFTLTISSLQPEDFATYYCQQLMSYPWTFGQGTKVEIKRTVAAPSVFIFPPSDEQLKSGTASVVCLLNNFYPREAKVQWKVDNALQSGNSQESVTEQDSKDSTYSLSSTLTLSKADYEKHKVYACEVTHQGLSSPVTKSFNRGEC

SEQ ID NO: 129 - protein, 214 aa, synthetic construct
DIQLTQSPSFLSASVGDRVTITCRASQGISSYLAWYQQKPGKAPKLLIYAASTLQSGVPSRFSGSGSGTEFTLTISSLQPEDFATYYCQQLQSYPWTFGQGTKVEIKRTVAAPSVFIFPPSDEQLKSGTASVVCLLNNFYPREAKVQWKVDNALQSGNSQESVTEQDSKDSTYSLSSTLTLSKADYEKHKVYACEVTHQGLSSPVTKSFNRGEC

SEQ ID NO: 130 - protein, 214 aa, synthetic construct
DIQLTQSPSFLSASVGDRVTITCRASQGISSYLAWYQQKPGKAPKLLIYAASTLQSGVPSRFSGSGSGTEFTLTISSLQPEDFATYYCQQLDSYPWTFGQGTKVEIKRTVAAPSVFIFPPSDEQLKSGTASVVCLLNNFYPREAKVQWKVDNALQSGNSQESVTEQDSKDSTYSLSSTLTLSKADYEKHKVYACEVTHQGLSSPVTKSFNRGEC

SEQ ID NO: 131 - protein, 214 aa, synthetic construct
DIQLTQSPSFLSASVGDRVTITCRASQGISSYLAWYQQKPGKAPKLLIYAASTLQSGVPSRFSGSGSGTEFTLTISSLQPEDFATYYCQQLGSYPWTFGQGTKVEIKRTVAAPSVFIFPPSDEQLKSGTASVVCLLNNFYPREAKVQWKVDNALQSGNSQESVTEQDSKDSTYSLSSTLTLSKADYEKHKVYACEVTHQGLSSPVTKSFNRGEC

SEQ ID NO: 132 - protein, 214 aa, synthetic construct
DIQLTQSPSFLSASVGDRVTITCRASQGISSYLAWYQQKPGKAPKLLIYAASTLQSGVPSRFSGSGSGTEFTLTISSLQPEDFATYYCQQLVSYPWTFGQGTKVEIKRTVAAPSVFIFPPSDEQLKSGTASVVCLLNNFYPREAKVQWKVDNALQSGNSQESVTEQDSKDSTYSLSSTLTLSKADYEKHKVYACEVTHQGLSSPVTKSFNRGEC

SEQ ID NO: 133 - protein, 214 aa, synthetic construct
DIQLTQSPSFLSASVGDRVTITCRASQGISSYLAWYQQKPGKAPKLLIYAASTLQSGVPSRFSGSGSGTEFTLTISSLQPEDFATYYCQQLNIYPWTFGQGTKVEIKRTVAAPSVFIFPPSDEQLKSGTASVVCLLNNFYPREAKVQWKVDNALQSGNSQESVTEQDSKDSTYSLSSTLTLSKADYEKHKVYACEVTHQGLSSPVTKSFNRGEC

SEQ ID NO: 134 - protein, 214 aa, synthetic construct
DIQLTQSPSFLSASVGDRVTITCRASQGISSYLAWYQQKPGKAPKLLIYAASTLQSGVPSRFSGSGSGTEFTLTISSLQPEDFATYYCQQLNFYPWTFGQGTKVEIKRTVAAPSVFIFPPSDEQLKSGTASVVCLLNNFYPREAKVQWKVDNALQSGNSQESVTEQDSKDSTYSLSSTLTLSKADYEKHKVYACEVTHQGLSSPVTKSFNRGEC

SEQ ID NO: 135 - protein, 214 aa, synthetic construct
DIQLTQSPSFLSASVGDRVTITCRASQGISSYLAWYQQKPGKAPKLLIYAASTLQSGVPSRFSGSGSGTEFTLTISSLQPEDFATYYCQQLNEYPWTFGQGTKVEIKRTVAAPSVFIFPPSDEQLKSGTASVVCLLNNFYPREAKVQWKVDNALQSGNSQESVTEQDSKDSTYSLSSTLTLSKADYEKHKVYACEVTHQGLSSPVTKSFNRGEC

SEQ ID NO: 136 - protein, 214 aa, synthetic construct
DIQLTQSPSFLSASVGDRVTITCRASQGISSYLAWYQQKPGKAPKLLIYAASTLQSGVPSRFSGSGSGTEFTLTISSLQPEDFATYYCQQLNLYPWTFGQGTKVEIKRTVAAPSVFIFPPSDEQLKSGTASVVCLLNNFYPREAKVQWKVDNALQSGNSQESVTEQDSKDSTYSLSSTLTLSKADYEKHKVYACEVTHQGLSSPVTKSFNRGEC

SEQ ID NO: 137 - protein, 214 aa, synthetic construct
DIQLTQSPSFLSASVGDRVTITCRASQGISSYLAWYQQKPGKAPKLLIYAASTLQSGVPSRFSGSGSGTEFTLTISSLQPEDFATYYCQQLNRYPWTFGQGTKVEIKRTVAAPSVFIFPPSDEQLKSGTASVVCLLNNFYPREAKVQWKVDNALQSGNSQESVTEQDSKDSTYSLSSTLTLSKADYEKHKVYACEVTHQGLSSPVTKSFNRGEC

SEQ ID NO: 138 - protein, 214 aa, synthetic construct
DIQLTQSPSFLSASVGDRVTITCRASQGISSYLAWYQQKPGKAPKLLIYAASTLQSGVPSRFSGSGSGTEFTLTISSLQPEDFATYYCQQLNNYPWTFGQGTKVEIKRTVAAPSVFIFPPSDEQLKSGTASVVCLLNNFYPREAKVQWKVDNALQSGNSQESVTEQDSKDSTYSLSSTLTLSKADYEKHKVYACEVTHQGLSSPVTKSFNRGEC

SEQ ID NO: 139 - protein, 214 aa, synthetic construct
DIQLTQSPSFLSASVGDRVTITCRASQGISSYLAWYQQKPGKAPKLLIYAASTLQSGVPSRFSGSGSGTEFTLTISSLQPEDFATYYCQQLNTYPWTFGQGTKVEIKRTVAAPSVFIFPPSDEQLKSGTASVVCLLNNFYPREAKVQWKVDNALQSGNSQESVTEQDSKDSTYSLSSTLTLSKADYEKHKVYACEVTHQGLSSPVTKSFNRGEC

SEQ ID NO: 140 - protein, 214 aa, synthetic construct
DIQLTQSPSFLSASVGDRVTITCRASQGISSYLAWYQQKPGKAPKLLIYAASTLQSGVPSRFSGSGSGTEFTLTISSLQPEDFATYYCQQLNQYPWTFGQGTKVEIKRTVAAPSVFIFPPSDEQLKSGTASVVCLLNNFYPREAKVQWKVDNALQSGNSQESVTEQDSKDSTYSLSSTLTLSKADYEKHKVYACEVTHQGLSSPVTKSFNRGEC

SEQ ID NO: 141 - protein, 214 aa, synthetic construct
DIQLTQSPSFLSASVGDRVTITCRASQGISSYLAWYQQKPGKAPKLLIYAASTLQSGVPSRFSGSGSGTEFTLTISSLQPEDFATYYCQQLNVYPWTFGQGTKVEIKRTVAAPSVFIFPPSDEQLKSGTASVVCLLNNFYPREAKVQWKVDNALQSGNSQESVTEQDSKDSTYSLSSTLTLSKADYEKHKVYACEVTHQGLSSPVTKSFNRGEC

SEQ ID NO: 142 - protein, 214 aa, synthetic construct
DIQLTQSPSFLSASVGDRVTITCRASQGISSYLAWYQQKPGKAPKLLIYAASTLQSGVPSRFSGSGSGTEFTLTISSLQPEDFATYYCQQLNMYPWTFGQGTKVEIKRTVAAPSVFIFPPSDEQLKSGTASVVCLLNNFYPREAKVQWKVDNALQSGNSQESVTEQDSKDSTYSLSSTLTLSKADYEKHKVYACEVTHQGLSSPVTKSFNRGEC

SEQ ID NO: 143 - protein, 214 aa, synthetic construct
DIQLTQSPSFLSASVGDRVTITCRASQGISSYLAWYQQKPGKAPKLLIYAASTLQSGVPSRFSGSGSGTEFTLTISSLQPEDFATYYCQQLNHYPWTFGQGTKVEIKRTVAAPSVFIFPPSDEQLKSGTASVVCLLNNFYPREAKVQWKVDNALQSGNSQESVTEQDSKDSTYSLSSTLTLSKADYEKHKVYACEVTHQGLSSPVTKSFNRGEC